European Patent Specification EP 3 612 208 B1, published April 5, 2023. Title: METHOD OF TREATMENT. Applicant: VOLUTION IMMUNO PHARMACEUTICALS SA. The sequence listing filed with the application follows.

SEQUENCE LISTING (29 sequences)

SEQ ID NO: 1 - DNA, 507 bp, Ornithodoros moubata
atgctggttttggtgaccctgattttctccttttctgcgaacatcgcatatgctgacagcgaaagcgactgcactggaagcgaacctgttgacgccttccaagctttcagtgagggcaaagaggcatatgtcctggtgaggtccacggatcccaaagcgagggactgcttgaaaggagaaccagccggagaaaagcaggacaacacgttgccggtgatgatgacgtttaagaatggcacagactgggcttcaaccgattggacgtttactttggacggcgcaaaggtaacggcaacccttggtaacctaacccaaaatagggaagtggtctacgactcgcaaagtcatcactgccacgttgacaaggtcgagaaggaagttccagattatgagatgtggatgctcgatgcgggagggcttgaagtggaagtcgagtgctgccgtcaaaagcttgaagagttggcgtctggcaggaaccaaatgtatccccatctcaaggactgctag

SEQ ID NO: 2 - protein, 168 aa, Ornithodoros moubata
MLVLVTLIFSFSANIAYADSESDCTGSEPVDAFQAFSEGKEAYVLVRSTDPKARDCLKGEPAGEKQDNTLPVMMTFKNGTDWASTDWTFTLDGAKVTATLGNLTQNREVVYDSQSHHCHVDKVEKEVPDYEMWMLDAGGLEVEVECCRQKLEELASGRNQMYPHLKDC

SEQ ID NO: 3 - DNA, 453 bp, Ornithodoros moubata
gacagcgaaagcgactgcactggaagcgaacctgttgacgccttccaagctttcagtgagggcaaagaggcatatgtcctggtgaggtccacggatcccaaagcgagggactgcttgaaaggagaaccagccggagaaaagcaggacaacacgttgccggtgatgatgacgtttaagaatggcacagactgggcttcaaccgattggacgtttactttggacggcgcaaaggtaacggcaacccttggtaacctaacccaaaatagggaagtggtctacgactcgcaaagtcatcactgccacgttgacaaggtcgagaaggaagttccagattatgagatgtggatgctcgatgcgggagggcttgaagtggaagtcgagtgctgccgtcaaaagcttgaagagttggcgtctggcaggaaccaaatgtatccccatctcaaggactgctag

SEQ ID NO: 4 - protein, 150 aa, Ornithodoros moubata
DSESDCTGSEPVDAFQAFSEGKEAYVLVRSTDPKARDCLKGEPAGEKQDNTLPVMMTFKNGTDWASTDWTFTLDGAKVTATLGNLTQNREVVYDSQSHHCHVDKVEKEVPDYEMWMLDAGGLEVEVECCRQKLEELASGRNQMYPHLKDC

SEQ ID NO: 5 - DNA, 450 bp, Ornithodoros moubata
agcgaaagcgactgcactggaagcgaacctgttgacgccttccaagctttcagtgagggcaaagaggcatatgtcctggtgaggtccacggatcccaaagcgagggactgcttgaaaggagaaccagccggagaaaagcaggacaacacgttgccggtgatgatgacgtttaagaatggcacagactgggcttcaaccgattggacgtttactttggacggcgcaaaggtaacggcaacccttggtaacctaacccaaaatagggaagtggtctacgactcgcaaagtcatcactgccacgttgacaaggtcgagaaggaagttccagattatgagatgtggatgctcgatgcgggagggcttgaagtggaagtcgagtgctgccgtcaaaagcttgaagagttggcgtctggcaggaaccaaatgtatccccatctcaaggactgctag

SEQ ID NO: 6 - protein, 149 aa, Ornithodoros moubata
SESDCTGSEPVDAFQAFSEGKEAYVLVRSTDPKARDCLKGEPAGEKQDNTLPVMMTFKNGTDWASTDWTFTLDGAKVTATLGNLTQNREVVYDSQSHHCHVDKVEKEVPDYEMWMLDAGGLEVEVECCRQKLEELASGRNQMYPHLKDC

SEQ ID NO: 7 - DNA, 447 bp, Ornithodoros moubata
gaaagcgactgcactggaagcgaacctgttgacgccttccaagctttcagtgagggcaaagaggcatatgtcctggtgaggtccacggatcccaaagcgagggactgcttgaaaggagaaccagccggagaaaagcaggacaacacgttgccggtgatgatgacgtttaagaatggcacagactgggcttcaaccgattggacgtttactttggacggcgcaaaggtaacggcaacccttggtaacctaacccaaaatagggaagtggtctacgactcgcaaagtcatcactgccacgttgacaaggtcgagaaggaagttccagattatgagatgtggatgctcgatgcgggagggcttgaagtggaagtcgagtgctgccgtcaaaagcttgaagagttggcgtctggcaggaaccaaatgtatccccatctcaaggactgctag

SEQ ID NO: 8 - protein, 148 aa, Ornithodoros moubata
ESDCTGSEPVDAFQAFSEGKEAYVLVRSTDPKARDCLKGEPAGEKQDNTLPVMMTFKNGTDWASTDWTFTLDGAKVTATLGNLTQNREVVYDSQSHHCHVDKVEKEVPDYEMWMLDAGGLEVEVECCRQKLEELASGRNQMYPHLKDC

SEQ ID NO: 9 - DNA, 444 bp, Ornithodoros moubata
agcgactgcactggaagcgaacctgttgacgccttccaagctttcagtgagggcaaagaggcatatgtcctggtgaggtccacggatcccaaagcgagggactgcttgaaaggagaaccagccggagaaaagcaggacaacacgttgccggtgatgatgacgtttaagaatggcacagactgggcttcaaccgattggacgtttactttggacggcgcaaaggtaacggcaacccttggtaacctaacccaaaatagggaagtggtctacgactcgcaaagtcatcactgccacgttgacaaggtcgagaaggaagttccagattatgagatgtggatgctcgatgcgggagggcttgaagtggaagtcgagtgctgccgtcaaaagcttgaagagttggcgtctggcaggaaccaaatgtatccccatctcaaggactgctag

SEQ ID NO: 10 - protein, 147 aa, Ornithodoros moubata
SDCTGSEPVDAFQAFSEGKEAYVLVRSTDPKARDCLKGEPAGEKQDNTLPVMMTFKNGTDWASTDWTFTLDGAKVTATLGNLTQNREVVYDSQSHHCHVDKVEKEVPDYEMWMLDAGGLEVEVECCRQKLEELASGRNQMYPHLKDC

SEQ ID NO: 11 - DNA, 441 bp, Ornithodoros moubata
gactgcactggaagcgaacctgttgacgccttccaagctttcagtgagggcaaagaggcatatgtcctggtgaggtccacggatcccaaagcgagggactgcttgaaaggagaaccagccggagaaaagcaggacaacacgttgccggtgatgatgacgtttaagaatggcacagactgggcttcaaccgattggacgtttactttggacggcgcaaaggtaacggcaacccttggtaacctaacccaaaatagggaagtggtctacgactcgcaaagtcatcactgccacgttgacaaggtcgagaaggaagttccagattatgagatgtggatgctcgatgcgggagggcttgaagtggaagtcgagtgctgccgtcaaaagcttgaagagttggcgtctggcaggaaccaaatgtatccccatctcaaggactgctag

SEQ ID NO: 12 - protein, 146 aa, Ornithodoros moubata
DCTGSEPVDAFQAFSEGKEAYVLVRSTDPKARDCLKGEPAGEKQDNTLPVMMTFKNGTDWASTDWTFTLDGAKVTATLGNLTQNREVVYDSQSHHCHVDKVEKEVPDYEMWMLDAGGLEVEVECCRQKLEELASGRNQMYPHLKDC

SEQ ID NO: 13 - DNA, 438 bp, Ornithodoros moubata
tgcactggaagcgaacctgttgacgccttccaagctttcagtgagggcaaagaggcatatgtcctggtgaggtccacggatcccaaagcgagggactgcttgaaaggagaaccagccggagaaaagcaggacaacacgttgccggtgatgatgacgtttaagaatggcacagactgggcttcaaccgattggacgtttactttggacggcgcaaaggtaacggcaacccttggtaacctaacccaaaatagggaagtggtctacgactcgcaaagtcatcactgccacgttgacaaggtcgagaaggaagttccagattatgagatgtggatgctcgatgcgggagggcttgaagtggaagtcgagtgctgccgtcaaaagcttgaagagttggcgtctggcaggaaccaaatgtatccccatctcaaggactgctag

SEQ ID NO: 14 - protein, 145 aa, Ornithodoros moubata
CTGSEPVDAFQAFSEGKEAYVLVRSTDPKARDCLKGEPAGEKQDNTLPVMMTFKNGTDWASTDWTFTLDGAKVTATLGNLTQNREVVYDSQSHHCHVDKVEKEVPDYEMWMLDAGGLEVEVECCRQKLEELASGRNQMYPHLKDC

SEQ ID NO: 15 - protein, 20 aa, Artificial Sequence
  PAS sequence
ASPAAPAPASPAAPAPSAPA

SEQ ID NO: 16 - protein, 20 aa, Artificial Sequence
  PAS sequence
AAPASPAPAAPSAPAPAAPS

SEQ ID NO: 17 - protein, 20 aa, Artificial Sequence
  PAS sequence
APSSPSPSAPSSPSPASPSS

SEQ ID NO: 18 - protein, 20 aa, Artificial Sequence
  PAS sequence
SAPSSPSPSAPSSPSPASPS

SEQ ID NO: 19 - protein, 20 aa, Artificial Sequence
  PAS sequence
SSPSAPSPSSPASPSPSSPA

SEQ ID NO: 20 - protein, 24 aa, Artificial Sequence
  PAS sequence
AASPAAPSAPPAAASPAAPSAPPA

SEQ ID NO: 21 - protein, 20 aa, Artificial Sequence
  PAS sequence
ASAAAPAAASAAASAPSAAA

SEQ ID NO: 22 - protein, 150 aa, Artificial Sequence
  Coversin variant 1
DSESDCTGSEPVDAFQAFSEGKEAYVLVRSTDPKARDCLKGEPAGEKQDNTLPVMMTFKNGTDWASTDWTFTLDGAKVTATLGNLTQNREVVYDSQSHHCHVDKVEKEVPDYEQWQSNGSADDKEVECCRQKLEELASGRNQMYPHLKDC

SEQ ID NO: 23 - protein, 150 aa, Artificial Sequence
  Coversin variant 2
DSESDCTGSEPVDAFQAFSEGKEAYVLVRSTDPKARDCLKGEPNGEKQDNTLPVMMTFKNGTDWASTDWTFTLDGAKVTATLGNLTQNREVVYDSQSHHCHVDKVEKEVPDYEMWQSDAGADAVEVECCRQKLEELASGRNQMYPHLKGC

SEQ ID NO: 24 - protein, 150 aa, Artificial Sequence
  Coversin variant 3
DSESDCTGSEPVDAFQAFSEGKEAYVLVRSTDPKARDCLKGEPNGEKQDNTLPVMMTFKNGTDWASTDWTFTLDGAKVTATLGNLTQNREVVYDSQSHHCHVDKVEKEVPDYEMWQLDAGGDEVEVECCRQKLEELASGRNQMYPHLKGC

SEQ ID NO: 25 - protein, 150 aa, Artificial Sequence
  Coversin variant 4
DSESDCTGSEPVDAFQAFSEGKEAYVLVRSTDPKARDCLKGEPNGEKQDNTLPVMMTFKNGTDWASTDWTFTLDGAKVTATLGNLTQNREVVYDSQSHHCHVDKVEKEVPDYEMWMLDAGGLEVEVECCRQKLEELASGRNQMYPHLKDC

SEQ ID NO: 26 - protein, 11 aa, Artificial Sequence
  Loop sequence
MWMLDAGGLEV

SEQ ID NO: 27 - protein, 11 aa, Artificial Sequence
  Loop sequence of Coversin variant 1
QWQSNGSADDK

SEQ ID NO: 28 - protein, 11 aa, Artificial Sequence
  Loop sequence of Coversin variant 2
MWQSDAGADAV

SEQ ID NO: 29 - protein, 11 aa, Loop sequence of Coversin variant 3
MWQLDAGGDEV